European Patent Specification EP 3 661 531 B1, published October 2, 2024. Title: LINEAR LIPOPEPTIDE PAENIPEPTINS AND METHODS OF USING THE SAME. Applicant: BioVentures, LLC HUANG, En MOON, Sun Hee SMELTZER, Mark MEEKER, Daniel. Application EP 18842362.8. The sequence listing filed with the application follows.

SEQUENCE LISTING (17 sequences)

SEQ ID NO: 1 - protein, 9 aa, Artificial Sequence
  Synthetic
  misc_feature (1)..(9): Xaa at positions 1, 3 and 6 is 2,4-diaminobutyric acid
  misc_feature (4)..(4): Phe is dPhe
  misc_feature (7)..(7): Val is dVal
XIXFLXVLS

SEQ ID NO: 2 - protein, 9 aa, Artificial Sequence
  Synthetic
  misc_feature (1)..(9): Xaa at positions 1, 3 and 6 is 2,4-diaminobutyric acid
  misc_feature (4)..(4): Phe is dPhe
  misc_feature (7)..(7): Val is dVal
XVXFLXVLS

SEQ ID NO: 3 - protein, 9 aa, Artificial Sequence
  Synthetic
  misc_feature (1)..(9): Xaa at positions 1, 3 and 6 is 2,4-diaminobutyric acid
  misc_feature (4)..(4): Phe is dPhe
  misc_feature (7)..(7): Val is dVal
XFXFLXVLS

SEQ ID NO: 4 - protein, 9 aa, Artificial Sequence
  Synthetic
  misc_feature (1)..(9): Xaa at positions 1, 3 and 6 is 2,4-diaminobutyric acid
  misc_feature (4)..(4): Phe is dPhe
  misc_feature (7)..(7): Leu is dLeu
XIXFLXLLS

SEQ ID NO: 5 - protein, 9 aa, Artificial Sequence
  Synthetic
  misc_feature (1)..(9): Xaa at positions 1, 3 and 6 is 2,4-diaminobutyric acid
  misc_feature (4)..(4): Phe is dPhe
  misc_feature (7)..(7): Leu is dLeu
XFXFLXLLS

SEQ ID NO: 6 - protein, 9 aa, Artificial Sequence
  Synthetic
  misc_feature (1)..(9): Xaa at positions 1, 3 and 6 is 2,4-diaminobutyric acid
  misc_feature (4)..(4): Phe is dPhe
  misc_feature (7)..(7): Leu is dLeu
XFXFLXLFS

SEQ ID NO: 7 - protein, 9 aa, Artificial Sequence
  Synthetic
  misc_feature (1)..(9): Xaa at positions 1, 3, 6 and 9 is 2,4-diaminobutyric acid
  misc_feature (4)..(4): Phe is dPhe
  misc_feature (7)..(7): Val is dVal
XIXFLXVLX

SEQ ID NO: 8 - protein, 9 aa, Artificial Sequence
  Synthetic
  misc_feature (1)..(9): Xaa at positions 1, 2, 3, 6 and 9 is 2,4-diaminobutyric acid
  misc_feature (4)..(4): Phe is dPhe
  misc_feature (7)..(7): Val is dVal
XXXFLXVLX

SEQ ID NO: 9 - protein, 9 aa, Artificial Sequence
  Synthetic
  misc_feature (1)..(9): Xaa at 1, 3, and 6 is ornithine
  misc_feature (4)..(4): Phe is dPhe
  misc_feature (7)..(7): Val is dVal
XIXFLXVLS

SEQ ID NO: 10 - protein, 9 aa, Artificial Sequence
  Synthetic
  misc_feature (1)..(9): Xaa at positions 1 and 6 is 2,4-diaminobutyric acid
  misc_feature (4)..(4): Leu is dLeu
  misc_feature (7)..(7): Val is dVal
XITLLXVLS

SEQ ID NO: 11 - protein, 9 aa, Artificial Sequence
  Synthetic
  misc_feature (1)..(9): Xaa at positions 1, 3 and 6 is 2,3-diaminopropionic acid
  misc_feature (4)..(4): Phe is dPhe
  misc_feature (7)..(7): Val is dVal
XIXFLXVLS

SEQ ID NO: 12 - protein, 9 aa, Artificial Sequence
  Synthetic
  misc_feature (1)..(9): Xaa at positions 1, 3 and 6 is 2,4-diaminobutyric acid
  misc_feature (2)..(2): Xaa is 4-phenyl-phenylalanyl
  misc_feature (4)..(4): Phe is dPhe
  misc_feature (7)..(7): Val is dVal
XXXFLXVLS

SEQ ID NO: 13 - protein, 9 aa, Artificial Sequence
  Synthetic
  misc_feature (1)..(9): Xaa at positions 1, 3 and 6 is 2,4-diaminobutyric acid
  misc_feature (4)..(4): Xaa is 4-phenyl-phenylalanyl
  misc_feature (7)..(7): Val is dVal
XIXXLXVLS

SEQ ID NO: 14 - protein, 9 aa, Artificial Sequence
  Synthetic
  misc_feature (1)..(9): Xaa at positions 1, 3 and 6 is 2,4-diaminobutyric acid
  misc_feature (4)..(4): Phe is dPhe
  misc_feature (5)..(5): Xaa is 4-phenyl-phenylalanyl
  misc_feature (7)..(7): Val is dVal
XIXFXXVLS

SEQ ID NO: 15 - protein, 9 aa, Artificial Sequence
  Synthetic
  misc_feature (1)..(9): Xaa at positions 1, 3 and 6 is 2,4-diaminobutyric acid
  misc_feature (4)..(4): Phe is dPhe
  misc_feature (7)..(7): Xaa is 4-phenyl-phenylalanyl
XIXFLXXLS

SEQ ID NO: 16 - protein, 9 aa, Artificial Sequence
  Synthetic
  misc_feature (1)..(9): Xaa at positions 1, 3 and 6 is 2,4-diaminobutyric acid
  misc_feature (4)..(4): Phe is dPhe
  misc_feature (7)..(7): Val is dVal
  misc_feature (8)..(8): Xaa is 4-phenyl-phenylalanyl
XIXFLXVXS

SEQ ID NO: 17 - protein, 9 aa, Artificial Sequence
  Synthetic
  misc_feature (1)..(9): Xaa at positions 1, 3 and 6 is 2,4-diaminobutyric acid
  misc_feature (4)..(4): Phe is dPhe
  misc_feature (7)..(7): Val is dVal
  misc_feature (8)..(8): Xaa is Octylglycy
XIXFLXVXS